European Patent Application EP 4 134 434 A1, published February 15, 2023. Title: Process for producing copolymerised polyhydroxyalkanoate mixture, and transformed microorganism. Applicant: Kaneka Corporation. The sequence listing filed with the application follows.

SEQUENCE LISTING (31 sequences)

SEQ ID NO: 1 - protein, 594 aa, Aeromonas caviae
MSQPSYGPLFEALAHYNDKLLAMAKAQTERTAQALLQTNLDDLGQVLEQGSQQPWQLIQAQMNWWQDQLKLMQHTLLKSAGQPSEPVITPERSDRRFKAEAWSEQPIYDYLKQSYLLTARHLLASVDALEGVPQKSRERLRFFTRQYVNAMAPSNFLATNPELLKLTLESDGQNLVRGLALLAEDLERSADQLNIRLTDESAFELGRDLALTPGRVVQRTELYELIQYSPTTETVGKTPVLIVPPFINKYYIMDMRPQNSLVAWLVAQGQTVFMISWRNPGVAQAQIDLDDYVVDGVIAALDGVEAATGEREVHGIGYCIGGTALSLAMGWLAARRQKQRVRTATLFTTLLDFSQPGELGIFIHEPIIAALEAQNEAKGIMDGRQLAVSFSLLRENSLYWNYYIDSYLKGQSPVAFDLLHWNSDSTNVAGKTHNSLLRRLYLENQLVKGELKIRNTRIDLGKVKTPVLLVSAVDDHIALWQGTWQGMKLFGGEQRFLLAESGHIAGIINPPAANKYGFWHNGAEAESPESWLAGATHQGGSWWPEMMGFIQNRDEGSEPVPARVPEEGLAPAPGHYVKVRLNPVFACPTEEDAA

SEQ ID NO: 2 - protein, 594 aa, Aeromonas caviae
MSQPSYGPLFEALAHYNDKLLAMAKAQTERTAQALLQTNLDDLGQVLEQGSQQPWQLIQAQMNWWQDQLKLMQHTLLKSAGQPSEPVITPERSDRRFKAEAWSEQPIYDYLKQSYLLTARHLLASVDALEGVPQKSRERLRFFTRQYVSAMAPSNFLATNPELLKLTLESGGQNLVRGLALLAEDLERSADQLNIRLTDESAFELGRDLALTPGRVVQRTELYELIQYSPTTETVGKTPVLIVPPFINKYYIMDMRPQNSLVAWLVAQGQTVFMISWRNPGVAQAQIDLDDYVVDGVIAALDGVEAATGEREVHGIGYCIGGTALSLAMGWLAARRQKQRVRTATLFTTLLDFSQPGELGIFIHEPIIAALEAQNEAKGIMDGRQLAVSFSLLRENSLYWNYYIDSYLKGQSPVAFDLLHWNSDSTNVAGKTHNSLLRRLYLENQLVKGELKIRNTRIDLGKVKTPVLLVSAVDDHIALWQGTWQGMKLFGGEQRFLLAESGHIAGIINPPAANKYGFWHNGAEAESPESWLAGATHQGGSWWPEMMGFIQNRDEGSEPVPARVPEEGLAPAPGHYVKVRLNPVFACPTEEDAA

SEQ ID NO: 3 - protein, 594 aa, Aeromonas caviae
MSQPSYGPLFEALAHYNDKLLAMAKAQTERTAQALLQTNLDDLGQVLEQGSQQPWQLIQAQMNWWQDQLKLMQHTLLKSAGQPSEPVITPERSDRRFKAEAWSEQPIYDYLKQSYLLTARHLLASVDALEGVPQKSRERLRFFTRQYVSAMAPSNFLATNPELLKLTLESGGQNLVRGLALLAEDLERSADQLNIRLTDESAFELGRDLALTPGRVVQRTELYELIQYSPTTETVGKTPVLIVPPFINKYYIMDMRPQNSLVAWLVAQGQTVFMISWRNPGVAQAQIDLDDYVVDGVIAALDGVEAATGEREVHGIGYCIGGTALSLAMGWLAARRQKQRVRTATLFTTLLDFSQPGELGIFIHEPIIAALEAQNEAKGIMDGRQLAVTFSLLRENSLYWNYYIDSYLKGQSPVAFDLLHWNSDSTNVAGKTHNSLLRRLYLENQLVKGELKIRNTRIDLGKVKTPVLLVSAVDDHIALWQGTWQGMKLFGGEQRFLLAESGHIAGIINPPAANKYGFWHNGAEAESPESWLAGATHQGGSWWPEMMGFIQNRDEGSEPVPARVPEEGLAPAPGHYVKVRLNPVFACPTEEDAA

SEQ ID NO: 4 - protein, 567 aa, Chromobacterium sp.
MQQFVNSLSLGQDQSDAPHPLTGAWSQLMSQTNQLLQLQSSLYQQQLGLWTQFLGQTAGNDASAPSAKPSDRRFASPEWDEHPFYSFLKQSYLQTSKWMMELVDKTQIDESAKDKLSFATRQYLDAMAPSNFMLTNPDVVKRAIETQGESLVEGMKNMMEDIQKGHISMSDESKFQIGKNLVVTPGEVVFRNELIELIQYTPTTEKVHEKPLLFVPPCINKYYLMDLQPDNSMVRHFVGQGYRVFLVSWRSAVPEMKNFTWETYIEKGVFAAAEAVQKITKQPTMNALGFCVGGVILTTALCVAQAKGLKYFDSATFMTSLIDHAEPGEISFFIDEALVASREAKMAAGGIISGKEIGRTFASLRANDLVWNYVVNNYLLGKTPAPFDLLYWNNDAVDLPLPMHTFMLRQFYINNALITPGAITLCGVPIDISKIDIPVYMFAAREDHIVLWSSAYSGLKYLSGTPSRRFVLGASGHIMGSINPVTKDKRNYWTNEQLPVNPEEWLEGAQSHPGSWWKDWDAWLAPQSGKQVPAPKMLGSKEFPPLQPAPGSYVLAKAMPPVAAALN

SEQ ID NO: 5 - protein, 567 aa, Chromobacterium sp.
MQQFVNSLSLGQDQSDAPHPLTGAWSQLMSQTNQLLQLQSSLYQQQLGLWTQFLGQTAGNDASAPSAKPSDRRFASPEWDEHPFYSFLKQSYLQTSKWMMELVDKTQIDESAKDKLSFATRQYLDAMAPSNFMLTNPDVVKRAIETQGESLVEGMKNMMEDIQKGHISMSDESKFQIGKNLVVTPGEVVFRNELIELIQYTPTTEKVHEKPLLFVPPCINKYYLMDLQPDNSMVRHFVGQGYRVFLVSWRSAVPEMKNFTWETYIEKGVFAAAEAVQKITKQPTMNALGFCVGGVILTTALCVAQAKGLKYFDSATFMTSLIDHAEPGEISFFIDEALVASREAKMAAGGIISGKEIGRTFASLRANDLVWNYVVNNYLLGKTPAPFDLLYWNNDAVDLPLPMHTFMLRQFYINNALITPGAITLCGVPIDISKIDIPVYMFAAREDHIVLWSSAYSGLKYLSGTPSRRFVLGASGHIGGSINPVTKDKRNYWTNEQLPVNPEEWLEGAQSHPGSWWKDWDAWLAPQSGKQVPAPKMLGSKEFPPLQPAPGSYVLAKAMPPVAAALN

SEQ ID NO: 6 - protein, 585 aa, Artificial
  Artificial
MSQPSYGPLFEALAHYNDKLLAMAKAQTERTAQALLQTNLDDLGQVLEQGSQQPWQLIQAQMNWWQDQLKLMQHTLLKSAGQPSEPVITPERSDRRFKAEAWSEQPIYDYLKQSYLLTARHLLASVDALEGVPQKSRERLRFFTRQYVSAMAPANFLATNPEAQRLLIESGGESLRAGVRNMMEDLTRGKISQTDESAFEVGRNVAVTEGAVVFENEYFQLLQYKPLTDKVHARPLLMVPPCINKYYILDLQPESSLVRHVVEQGHTVFLVSWRNPDASMAGSTWDDYIEHAAIRAIEVARDISGQDKINVLGFCVGGTIVSTALAVLAARGEHPAASVTLLTTLLDFADTGILDVFVDEGHVQLREATLGGGAGAPCALLRGLELANTFSFLRPNDLVWNYVVDNYLKGNTPVPFDLLFWNGDATNLPGPWYCWYLRHTYLQNELKVPGKLTVCGVPVDLASIDVPTYIYGSREDHIVPWTAAYASTALLANKLRFVLGASGHIAGVINPPAKNKRSHWTNDALPESPQQWLAGAIEHHGSWWPDWTAWLAGQAGAKRAAPANYGNARYRAIEPAPGRYVKAKA

SEQ ID NO: 7 - protein, 160 aa, Bacillus cereus
MIDQKFDPLQAWKNAYEQTETFWGKALNETIKTEEYSAWMGSVLDLNLFYQKALNDTTKNYLEQVNVPTKEDIARVATLVINLENKVDNIEEFLEEKVESVGQAPTLKRDVTKVKQDIRTLETKVDQILELLEKQNAVLAKLQEPVKEEVKPTNKPENKK

SEQ ID NO: 8 - protein, 361 aa, Bacillus cereus
MTTFATEWEKQLELYPEEYRKAYRRVKRASEILLREPEPQVGLTPKEVIWTKNKTKLYRYIPKQEKTQRVPILLIYALINKPYIMDLTPGNSLVEYLVDRGFDVYMLDWGTFGLEDSHLKFDDFVFDYIAKAVKKVMRTAKSDEISLLGYCMGGTLTSIYAALHPHMPIRNLIFMTSPFDFSETGLYGPLLDEKYFNLDKAVDTFGNIPPEMIDFGNKMLKPITNFVGPYVALVDRSENERFVESWRLVQKWVGDGIPFPGESYRQWIRDFYQNNKLVKGELVIRGQKVDLANIKANVLNISGKRDHIALPCQVEALLDHISSTDKQYVCLPTGHMSIVYGGTAVKQTYPTIGNWLEERSN

SEQ ID NO: 9 - protein, 394 aa, Cupriavidus necator
MTREVVVVSGVRTAIGTFGGSLKDVAPAELGALVVREALARAQVSGDDVGHVVFGNVIQTEPRDMYLGRVAAVNGGVTINAPALTVNRLCGSGLQAIVSAAQTILLGDTDVAIGGGAESMSRAPYLAPAARWGARMGDAGLVDMMLGALHDPFHRIHMGVTAENVAKEYDISRAQQDEAALESHRRASAAIKAGYFKDQIVPVVSKGRKGDVTFDTDEHVRHDATIDDMTKLRPVFVKENGTVTAGNASGLNDAAAAVVMMERAEAERRGLKPLARLVSYGHAGVDPKAMGIGPVPATKIALERAGLQVSDLDVIEANEAFAAQACAVTKALGLDPAKVNPNGSGISLGHPIGATGALITVKALHELNRVQGRYALVTMCIGGGQGIAAIFERI

SEQ ID NO: 10 - protein, 392 aa, Cupriavidus necator
MNEAVIVSTARTPLAKSWKGAFNMTHGATLGGHAVQHAIARAKIEAAEVEDVLMGCANPEGATGANIARQIALRAGCPVTVPGATVNRFCSSGLQTIAMAAQRVIADEGDIFVAGGVESISCVQQEMNRHMVQESWLLKNKPEIYWNMLQTAENVAKRYNISKERQDEYGVRSQQRAAAGQEAGKFKDEIVPMTVLAGVADKSTGQLVTKEVTVSADEGIRADTTLEGVSKIRSAVPGGVITAGNASQFSDGASAAVVMNARVAEARGLQPLGVFRGFAVAGCEPDEMGIGPVFAVPKLLKKAGLKVDDIGLWELNEAFAVQVLYCADTLGIPMDRLNVNGGAIAVGHPYGVSGARLVGHALIEGKRRGVKYVVVTMCIGGGQGAAGLFEVL

SEQ ID NO: 11 - protein, 134 aa, Aeromonas caviae
MSAQSLEVGQKARLSKRFGAAEVAAFAALSEDFNPLHLDPAFAATTAFERPIVHGMLLASLFSGLLGQQLPGKGSIYLGQSLSFKLPVFVGDEVTAEVEVTALREDKPIATLTTRIFTQGGALAVTGEAVVKLP

SEQ ID NO: 12 - protein, 158 aa, Cupriavidus necator
MRTIASLEELEGLQGQEVAVSDWIEVTQQQVNQFADATGDHQWIHIDVERAKKESPYGGPIAHGFLTLSLLPKFMHNALHMPSKIGVNYGLNRVRFTAPVPVGSKLRARIKLLKVERLDPLPKSPELVGAQSTWEVTVEREGSDRPVCVAESITRRYG

SEQ ID NO: 13 - protein, 151 aa, Cupriavidus necator
MKTYENIADLQPLVGEVIGTSEWLALDQARINTFADATGDHQWIHVDVERAKNGPFGAPIAHGFLTLSLLPAFTHSAYRIRNSSTGVNYGLDKVRFPAPVPVDSLLRAQFKLMSYEALENGGAQFKVEMMVERQGGSKPVCIAESILRRFP

SEQ ID NO: 14 - protein, 901 aa, Yarrowia lipolytica
MSGELRYDGKVVIVTGAGGGLGKAYALFYGSRGASVVVNDLGGDFKGDGAQAGSGKRVADVVVDEIVSKGGKAVANYDSVENGDKIVETAVKAFGSVHIVINNAGILRDISFKKMTDKDWDLVYKVHVFGAYKVTRAAWPYFRKQKYGRVISTSSAAGLYGNFGQTNYSAAKLALVGFGETLAKEGAKYNITSNVIAPLAASRMTETVMPEDILKLLKPEYVVPLVGYLTHDSVTESYGIYEVGAGYMAKIRWERGNGAVFKGDDTFTPSAILKRWDEVTSFESPTYPNGPADFFKYAEESVKRPENPQGPTVSFKDQVVIVTGAGAGIGRAYSHLLAKLGAKVVVNDFGNPQKVVDEIKALGGIAVADKNNVIHGEKVVQTAIDAFGAVHAVVNNAGILRDKSFANMDDEMWQLIFDVHLNGTYSVTKAAWPHFLKQKYGRVINTTSTSGIYGNFGQANYSAAKAGILGFSRALAREGEKYNILVNTIAPNAGTAMTASVFTEEMLELFKPDFIAPITVLLASDQAPVTGDLFETGSAWIGQTRWQRAGGKAFNTKKGVTPEMVRDSWAKIVDFDDGNSTHPTTPSESTTQILENIFNVPDEEVEETALVAGPGGPGILNKEGEPFDYTYTYRDLILYNLGLGAKANELKYVFEGDDDFQTVPTFGVIPYMGGLITTNYGDFVPNFNPMMLLHGEQYLEIRQWPIPTNATLENKAKVIDVVDKGKAALLVTATTTTNKETGEEVFYNESSLFIRGSGGFGGKSTGTDRGAATAANKPPARAPDFVKEIKIQEDQAAIYRLSGDYNPLHIDPAFAAVGNFDRPILHGLCSFGVSGKALYDQFGPFKNAKVRFAGHVFPGETLKVEGWKEGNKVIFQTKVVERGTTAISNAAIELFPKDAKL

SEQ ID NO: 15 - protein, 598 aa, Drosophila melanogaster
MSSSDGKLRYDGRVAVVTGAGAGLGREYALLFAERGAKVVVNDLGGTHSGDGASQRAADIVVDEIRKAGGEAVADYNSVIDGAKVIETAIKAFGRVDILVNNAGILRDRSLVKTSEQDWNLVNDVHLKGSFKCTQAAFPYMKKQNYGRIIMTSSNSGIYGNFGQVNYTAAKMGLIGLANTVAIEGARNNVLCNVIVPTAASRMTEGILPDILFNELKPKLIAPVVAYLCHESCEDNGSYIESAAGWATKLHMVRGKGAVLRPSLDDPVTIEYVKDVWSNVTDMSKAKHLGAIAEASGTLLEVLEKLKEGGGDAIEDAFEFNSKELITYALGIGASVKNAKDMRFLYENDADFAAIPTFFVLPGLLLQMSTDKLLSKALPNSQVDFSNILHGEQYLEIVDDLPTSGTLLTNGKVFDVMDKGSGAVVVTNSESFDESGRLLVRNQSTTFIVGAGKFGGKKDPIAGVVPLQPAPNRQPDATVQYTTSEDQAALYRLSGDKNPLHIDPQMALLAGFKTPILHGLCTLGFSVRAVLAQFADNNPALFKAVKVRFSGPVIPGQTLRVDLWKQGTRINFRTVVVETGKEVISGAYVDLKSSQAKL

SEQ ID NO: 16 - DNA, 29 bp, Escherichia coli
tttacacttatgcttccggctcgtatgtt

SEQ ID NO: 17 - DNA, 31 bp, Escherichia coli
tttacacctttatgcttccggctcgtatgtt

SEQ ID NO: 18 - DNA, 1056 bp, Artificial
  Artificial
gcgcgcatttaaatctgccaccacgttgtgctcggtgatcgccatcatcagcgccacgtagagccagccaatggccacgatgtacatcaaaaattcatccttctcgcctatgctctggggcctcggcagatgcgagcgctgcataccgtccggtaggtcgggaagcgtgcagtgccgaggcggattcccgcattgacagcgcgtgcgttgcaaggcaacaatggactcaaatgtctcggaatcgctgacgattcccaggtttctccggcaagcatagcgcatggcgtctccatgcgagaatgtcgcgcttgccggataaaaggggagccgctatcggaatggacgcaagccacggccgcagcaggtgcggtcgagggcttccagccagttccagggcagatgtgccggcagaccctcccgctttgggggaggcgcaagccgggtccattcggatagcatctccccatgcaaagtgccggccagggcaatgcccggagccggttcgaatagtgacggcagagagacaatcaaatccgcttgcatgagtgccggcgtgcgtcatgcacagcgccggcaggcctgcaggttccctcccgtttccattgaaaggactacacaatgactgacgttgtcatcgtatccgccgcccgcaccgcggtcggcaagtttggcggctcgctggccaagatcccggcaccggaactgggtgccgtggtcatcaaggccgcgctggagcgcgccggcgtcaagccggagcaggtgagcgaagtcatcatgggccaggtgctgaccgccggttcgggccagaaccccgcacgccaggccgcgatcaaggccggcctgccggcgatggtgccggccatgaccatcaacaaggtgtgcggctcgggcctgaaggccgtgatgctggccgccaacgcgatcatggcgggcgacgccgagatcgtggtggccggcggccaggaaaacatgagcgccgccccgcacgtgctgccgggctcgcgcgatggtttccgcatgggcgatgccaagctggtcgacaatttaaatgcgcgc

SEQ ID NO: 19 - DNA, 3034 bp, Artificial
  Artificial
tacgctagcgtaccgagctatccatttaaatggagttccagaccctgctcgactttatcgccgaagccgaactggaccgcgtcggctgcttcgcctactcgccggtggagggcgccaccgccaatgacctgccgggcgcgctgcccgacgaggtgcgcgaggaacgccgcgcccgcttcatggaagtggccgaagaggtctcggcgcgccgcctgcagcgcaaggtcggccagaccctgcgcgtgctggtggacgaggtcaaccaggatggcggcatcggccgttcgtccgcggatgcgccggaaatcgacggcctcgtctatatcgcgccgccggaacgccacgcccagcgctatcgcgccggcgagttcgtcgacgtgaagatcaccggcgccgatggccacgacctgtggggcgcggtctgaaacgggttgattaggtaaaagtacgctcgttcgatttcgtccgcgtcccgctatactgtgcggtgcaacataacctcatggagacaaagtccaattggcgcaacgcaattaatgtgagttagctcactcattaggcaccccaggctttacacctttatgcttccggctcgtatgttgtgtggaattgtgagcggataacaatttcacacaggaaacaattgcacgtgcagagagacaatcaaatcatgagccaaccatcttatggcccgctgttcgaggccctggcccactacaatgacaagctgctggccatggccaaggcccagacagagcgcaccgcccaggcgctgctgcagaccaatctggacgatctgggccaggtgctggagcagggcagccagcaaccctggcaactgatccaggcccagatgaactggtggcaggatcagctcaagctgatgcagcacaccctgctcaaaagcgcaggccagccgagcgagccggtgatcaccccggagcgcagcgatcgccgcttcaaggccgaggcctggagcgaacaacccatctatgactacctcaagcagtcctacctgctcaccgccaggcacctgctggcctcggtggatgccctggagggcgtcccccagaagagccgggagcggctgcgtttcttcacccgccagtacgtcagcgccatggcccccagcaacttcctggccaccaaccccgagctgctcaagctgaccctggagtccggcggccagaacctggtgcgcgggctggccctcttggccgaggatctggagcgcagcgccgatcagctcaacatccgcctgaccgacgaatccgccttcgagctcgggcgggatctggcgctcaccccgggccgggtggtgcagcgcaccgagctctatgagctgatccagtacagcccgactaccgagacggtgggcaagacacctgtgctgatagtgccccccttcatcaacaagtactacatcatggacatgcggccccagaactccctggtcgcctggctggtcgcccagggccagacggtgttcatgatctcctggcgcaacccgggcgtggcccaggcccaaatcgatctcgacgactacgtggtggacggggtcatcgccgccctggacggggtggaggcggccaccggcgagcgggaggtgcacggcatcggctactgcatcggcggcactgcactgtcgctcgccatgggctggctggcggcgcggcgccagaagcagcgagtgcgcaccgccaccctgttcactaccctgctggacttctcccagccaggggagctcggcatcttcatccacgagcccatcatagcggcgctcgaggcgcaaaatgaggccaagggcatcatggacgggcgccagctggctgtctccttcagcctgctgcgggagaacagcctctactggaactactacatcgacagctacctcaagggccagagcccggtggccttcgatctgctgcactggaacagcgacagcaccaatgtggcgggcaagacccacaacagcctgctgcgccgtctctacctggagaaccagctggtgaagggggagctcaagatccgcaacacccgcatcgatctcggcaaggtgaaaaccccggtactgctggtgtcggccgtggacgatcacatcgccctctggcagggcacctggcagggcatgaagctgtttggcggggagcagcgcttcctcctggcggagtccggccacatcgccggcatcatcaacccgccggccgccaacaagtacggcttctggcacaacggggccgaggccgagagcccggagagctggctggcaggggcgacgcaccagggcggctcctggtggcccgagatgatgggctttatccagaaccgtgacgaagggtcggagcccgtccccgcgcgggtgcccgaggaggggctggcccccgcccccggccactatgtcaaggtgcggctcaaccccgtgtttgcctgcccaacagaggaggacgccgcatgacctgccggcctggttcaaccagtcggcagccgactagtggttagccttgcgccttgcttcgctgacgaagaacctctgcgcgctcggcctggccgccgtgctcgcgctggcgggcacggcgcaggcagcgccggcgaccgagctgtcgaccggcccggttaacaccgggccagccggcggcgaaggcctgggcatcaaccaggccattcgcgacggcgaagcccggcgcggcggcacctcgctttccactggcgcgccaaaacccctggcgccgcggccggaatatgcgtcgctgccggtctacgtcggcaaggtcggcgaccagccggtgcggctgcgcctgggccccaagcctgacgagcgcgacagcgtgcgtggcgaatacgccggccgtggcgccggtgtgcgcctgctggcaggcgagtgggaggacggcgccttcctgatggaggagtccgacgacggcacccgcgtatcgggcaactgggaaggcagcatcgacgccagcggcgccgtgcgcggcacctggaccgaatttaaatccgaattcactggccgtcgttttacaacgtcgtgact

SEQ ID NO: 20 - DNA, 2825 bp, Artificial
  Artificial
tacgctagcgtaccgagctatccatttaaattgcatgcgggcttgcacgtgccgcatgcgcggctggtgatccgcaagggccaccatgccgacgtggacagctactccgccttcctggaggcggaccgcaccacgcgcaccgggctggccggctacctgcgcgagcatggcgtcaggcgcgtgttctgcgcgggtctggcgacggactactgcgtggcctggagcgcgctcgatgcacgcgccgcgggcttcgcggccgcggtgatcgaggatgcctgccgcgccatcgacctggaagggtcgctggccaaagcatggcaggacctcggcgccgccggcgttgcgcgcgtcacgtccgctgaactgctcaagggccagggctgaaccgaaccaccgaactgaacgacacaagagaatccgaggagcaagaccaattggcgcaacgcaattaatgtgagttagctcactcattaggcaccccaggctttacacttatgcttccggctcgtatgttgtgtggaattgtgagcggataacaatttcacacaggaaacaattgcacgtgcagagagacaatcaaatcatgagccaaccatcttatggcccgctgttcgaggccctggcccactacaatgacaagctgctggccatggccaaggcccagacagagcgcaccgcccaggcgctgctgcagaccaatctggacgatctgggccaggtgctggagcagggcagccagcaaccctggcagctgatccaggcccagatgaactggtggcaggatcagctcaagctgatgcagcacaccctgctcaaaagcgcaggccagccgagcgagccggtgatcaccccggagcgcagcgatcgccgcttcaaggccgaggcctggagcgaacaacccatctatgactacctcaagcagtcctacctgctcaccgccaggcacctgctggcctcggtggatgccctggagggcgtcccccagaagagccgggagcggctgcgtttcttcacccgccagtacgtcagcgccatggcccccgccaacttccttgccaccaatcccgaggcgcagcgcctgctgatcgagtcgggcggcgaatcgctgcgtgccggcgtgcgcaacatgatggaagacctgacacgcggcaagatctcgcagaccgacgagagcgcgtttgaggtcggccgcaatgtcgcggtgaccgaaggcgccgtggtcttcgagaacgagtacttccagctgttgcagtacaagccgctgaccgacaaggtgcacgcgcgcccgctgctgatggtgccgccgtgcatcaacaagtactacatcctggacctgcagccggagagctcgctggtgcgccatgtggtggagcagggacatacggtgtttctggtgtcgtggcgcaatccggacgccagcatggccggcagcacctgggacgactacatcgagcacgcggccatccgcgccatcgaagtcgcgcgcgacatcagcggccaggacaagatcaacgtgctcggcttctgcgtgggcggcaccattgtctcgaccgcgctggcggtgctggccgcgcgcggcgagcacccggccgccagcgtcacgctgctgaccacgctgctggactttgccgacacgggcatcctcgacgtctttgtcgacgagggccatgtgcagttgcgcgaggccacgctgggcggcggcgccggcgcgccgtgcgcgctgctgcgcggccttgagctggccaataccttctcgttcttgcgcccgaacgacctggtgtggaactacgtggtcgacaactacctgaagggcaacacgccggtgccgttcgacctgctgttctggaacggcgacgccaccaacctgccggggccgtggtactgctggtacctgcgccacacctacctgcagaacgagctcaaggtaccgggcaagctgaccgtgtgcggcgtgccggtggacctggccagcatcgacgtgccgacctatatctacggctcgcgcgaagaccatatcgtgccgtggaccgcggcctatgcctcgaccgcgctgctggcgaacaagctgcgcttcgtgctgggtgcgtcgggccatatcgccggtgtgatcaacccgccggccaagaacaagcgcagccactggactaacgatgcgctgccggagtcgccgcagcaatggctggccggcgccatcgagcatcacggcagctggtggccggactggaccgcatggctggccgggcaggccggcgcgaaacgcgccgcgcccgccaactatggcaatgcgcgctatcgcgcaatcgaacccgcgcctgggcgatacgtcaaagccaaggcatgacctgccggcctggttcaaccagtcggcagccgactagtatgtcggctgcgggcaccgcgcgggccacgcccgccgacatgctcgcctggggccgggaggtgctggccagccagcccttctcggtcctggtcggcaccgaactggcggcgttgtcgccgggcaaggctgagttgcgcctgccgatccgtcaggacctgcggcagcagcacggcttcctgcacggcggcgtggtcagctacctggccgacaatgcgctgacctacgcgggcggcgcggccatggcggtgccggtcgtgacatccgagtacaagatcaactacgtgcgcccggcgatcggcgagctgctggtcgcccgcgccgaatgcgtcagcgccggccgccagcaggcggtggtgcgctgcgacgtgtacgtcgtcagggatggcgaggagaggctctgatttaaatccgaattcactggccgtcgttttacaacgtcgtgact

SEQ ID NO: 21 - DNA, 3033 bp, Artificial
  Artificial
tacgctagcgtaccgagctatccatttaaatggagttccagaccctgctcgactttatcgccgaagccgaactggaccgcgtcggctgcttcgcctactcgccggtggagggcgccaccgccaatgacctgccgggcgcgctgcccgacgaggtgcgcgaggaacgccgcgcccgcttcatggaagtggccgaagaggtctcggcgcgccgcctgcagcgcaaggtcggccagaccctgcgcgtgctggtggacgaggtcaaccaggatggcggcatcggccgttcgtccgcggatgcgccggaaatcgacggcctcgtctatatcgcgccgccggaacgccacgcccagcgctatcgcgccggcgagttcgtcgacgtgaagatcaccggcgccgatggccacgacctgtggggcgcggtctgaaacgggttgattaggtaaaagtacgctcgttcgatttcgtccgcgtcccgctatactgtgcggtgcaacataacctcatggagacaaagtccaattggcgcaacgcaattaatgtgagttagctcactcattaggcaccccaggctttacactttatgcttccggctcgtatgttgtgtggaattgtgagcggataacaatttcacacaggaaacaattgcacgtgcagagagacaatcaaatcatgagccaaccatcttatggcccgctgttcgaggccctggcccactacaatgacaagctgctggccatggccaaggcccagacagagcgcaccgcccaggcgctgctgcagaccaatctggacgatctgggccaggtgctggagcagggcagccagcaaccctggcaactgatccaggcccagatgaactggtggcaggatcagctcaagctgatgcagcacaccctgctcaaaagcgcaggccagccgagcgagccggtgatcaccccggagcgcagcgatcgccgcttcaaggccgaggcctggagcgaacaacccatctatgactacctcaagcagtcctacctgctcaccgccaggcacctgctggcctcggtggatgccctggagggcgtcccccagaagagccgggagcggctgcgtttcttcacccgccagtacgtcagcgccatggcccccagcaacttcctggccaccaaccccgagctgctcaagctgaccctggagtccggcggccagaacctggtgcgcgggctggccctcttggccgaggatctggagcgcagcgccgatcagctcaacatccgcctgaccgacgaatccgccttcgagctcgggcgggatctggcgctcaccccgggccgggtggtgcagcgcaccgagctctatgagctgatccagtacagcccgactaccgagacggtgggcaagacacctgtgctgatagtgccccccttcatcaacaagtactacatcatggacatgcggccccagaactccctggtcgcctggctggtcgcccagggccagacggtgttcatgatctcctggcgcaacccgggcgtggcccaggcccaaatcgatctcgacgactacgtggtggacggggtcatcgccgccctggacggggtggaggcggccaccggcgagcgggaggtgcacggcatcggctactgcatcggcggcactgcactgtcgctcgccatgggctggctggcggcgcggcgccagaagcagcgagtgcgcaccgccaccctgttcactaccctgctggacttctcccagccaggggagctcggcatcttcatccacgagcccatcatagcggcgctcgaggcgcaaaatgaggccaagggcatcatggacgggcgccagctggctgtctccttcagcctgctgcgggagaacagcctctactggaactactacatcgacagctacctcaagggccagagcccggtggccttcgatctgctgcactggaacagcgacagcaccaatgtggcgggcaagacccacaacagcctgctgcgccgtctctacctggagaaccagctggtgaagggggagctcaagatccgcaacacccgcatcgatctcggcaaggtgaaaaccccggtactgctggtgtcggccgtggacgatcacatcgccctctggcagggcacctggcagggcatgaagctgtttggcggggagcagcgcttcctcctggcggagtccggccacatcgccggcatcatcaacccgccggccgccaacaagtacggcttctggcacaacggggccgaggccgagagcccggagagctggctggcaggggcgacgcaccagggcggctcctggtggcccgagatgatgggctttatccagaaccgtgacgaagggtcggagcccgtccccgcgcgggtgcccgaggaggggctggcccccgcccccggccactatgtcaaggtgcggctcaaccccgtgtttgcctgcccaacagaggaggacgccgcatgacctgccggcctggttcaaccagtcggcagccgactagtggttagccttgcgccttgcttcgctgacgaagaacctctgcgcgctcggcctggccgccgtgctcgcgctggcgggcacggcgcaggcagcgccggcgaccgagctgtcgaccggcccggttaacaccgggccagccggcggcgaaggcctgggcatcaaccaggccattcgcgacggcgaagcccggcgcggcggcacctcgctttccactggcgcgccaaaacccctggcgccgcggccggaatatgcgtcgctgccggtctacgtcggcaaggtcggcgaccagccggtgcggctgcgcctgggccccaagcctgacgagcgcgacagcgtgcgtggcgaatacgccggccgtggcgccggtgtgcgcctgctggcaggcgagtgggaggacggcgccttcctgatggaggagtccgacgacggcacccgcgtatcgggcaactgggaaggcagcatcgacgccagcggcgccgtgcgcggcacctggaccgaatttaaatccgaattcactggccgtcgttttacaacgtcgtgact

SEQ ID NO: 22 - DNA, 140 bp, Artificial
  Artificial
gcgcgcgaattcgcgcaacgcaattaatgtgagttagctcactcattaggcaccccaggctttacacttatgcttccggctcgtatgttgtgtggaattgtgagcggataacaatttcacacaggaaacaattggcgcgc

SEQ ID NO: 23 - DNA, 3706 bp, Artificial
  Artificial
ggaaacaattgcacgtgcagagagacaatcaaatcatgagccaaccatcttatggcccgctgttcgaggccctggcccactacaatgacaagctgctggccatggccaaggcccagacagagcgcaccgcccaggcgctgctgcagaccaatctggacgatctgggccaggtgctggagcagggcagccagcaaccctggcagctgatccaggcccagatgaactggtggcaggatcagctcaagctgatgcagcacaccctgctcaaaagcgcaggccagccgagcgagccggtgatcaccccggagcgcagcgatcgccgcttcaaggccgaggcctggagcgaacaacccatctatgactacctcaagcagtcctacctgctcaccgccaggcacctgctggcctcggtggatgccctggagggcgtcccccagaagagccgggagcggctgcgtttcttcacccgccagtacgtcagcgccatggcccccgccaacttccttgccaccaatcccgaggcgcagcgcctgctgatcgagtcgggcggcgaatcgctgcgtgccggcgtgcgcaacatgatggaagacctgacacgcggcaagatctcgcagaccgacgagagcgcgtttgaggtcggccgcaatgtcgcggtgaccgaaggcgccgtggtcttcgagaacgagtacttccagctgttgcagtacaagccgctgaccgacaaggtgcacgcgcgcccgctgctgatggtgccgccgtgcatcaacaagtactacatcctggacctgcagccggagagctcgctggtgcgccatgtggtggagcagggacatacggtgtttctggtgtcgtggcgcaatccggacgccagcatggccggcagcacctgggacgactacatcgagcacgcggccatccgcgccatcgaagtcgcgcgcgacatcagcggccaggacaagatcaacgtgctcggcttctgcgtgggcggcaccattgtctcgaccgcgctggcggtgctggccgcgcgcggcgagcacccggccgccagcgtcacgctgctgaccacgctgctggactttgccgacacgggcatcctcgacgtctttgtcgacgagggccatgtgcagttgcgcgaggccacgctgggcggcggcgccggcgcgccgtgcgcgctgctgcgcggccttgagctggccaataccttctcgttcttgcgcccgaacgacctggtgtggaactacgtggtcgacaactacctgaagggcaacacgccggtgccgttcgacctgctgttctggaacggcgacgccaccaacctgccggggccgtggtactgctggtacctgcgccacacctacctgcagaacgagctcaaggtaccgggcaagctgaccgtgtgcggcgtgccggtggacctggccagcatcgacgtgccgacctatatctacggctcgcgcgaagaccatatcgtgccgtggaccgcggcctatgcctcgaccgcgctgctggcgaacaagctgcgcttcgtgctgggtgcgtcgggccatatcgccggtgtgatcaacccgccggccaagaacaagcgcagccactggactaacgatgcgctgccggagtcgccgcagcaatggctggccggcgccatcgagcatcacggcagctggtggccggactggaccgcatggctggccgggcaggccggcgcgaaacgcgccgcgcccgccaactatggcaatgcgcgctatcgcgcaatcgaacccgcgcctgggcgatacgtcaaagccaaggcatgacgctttaaagagtgccggcgtgcgtcatgcacggcgccggcaggcctgcaggttccctcccgtttccattgaaaggactacacaatgagccaaccatcttatggcccgctgttcgaggccctggcccactacaatgacaagctgctggccatggccaaggcccagacagagcgcaccgcccaggcgctgctgcagaccaatctggacgatctgggccaggtgctggagcagggcagccagcaaccctggcagctgatccaggcccagatgaactggtggcaggatcagctcaagctgatgcagcacaccctgctcaaaagcgcaggccagccgagcgagccggtgatcaccccggagcgcagcgatcgccgcttcaaggccgaggcctggagcgaacaacccatctatgactacctcaagcagtcctacctgctcaccgccaggcacctgctggcctcggtggatgccctggagggcgtcccccagaagagccgggagcggctgcgtttcttcacccgccagtacgtcagcgccatggcccccagcaacttcctggccaccaaccccgagctgctcaagctgaccctggagtccggcggccagaacctggtgcgcggactggccctcttggccgaggatctggagcgcagcgccgatcagctcaacatccgcctgaccgacgaatccgccttcgagctcgggcgggatctggccctgaccccgggccgggtggtgcagcgcaccgagctctatgagctcattcagtacagcccgactaccgagacggtgggcaagacacctgtgctgatagtgccgcccttcatcaacaagtactacatcatggacatgcggccccagaactccctggtcgcctggctggtcgcccagggccagacggtattcatgatctcctggcgcaacccgggcgtggcccaggcccaaatcgatctcgacgactacgtggtggatggcgtcatcgccgccctggacggcgtggaggcggccaccggcgagcgggaggtgcacggcatcggctactgcatcggcggcaccgccctgtcgctcgccatgggctggctggcggcgcggcgccagaagcagcgggtgcgcaccgccaccctgttcactaccctgctggacttctcccagcccggggagcttggcatcttcatccacgagcccatcatagcggcgctcgaggcgcaaaatgaggccaagggcatcatggacgggcgccagctggcggtctccttcagcctgctgcgggagaacagcctctactggaactactacatcgacagctacctcaagggtcagagcccggtggccttcgatctgctgcactggaacagcgacagcaccaatgtggcgggcaagacccacaacagcctgctgcgccgtctctacctggagaaccagctggtgaagggggagctcaagatccgcaacacccgcatcgatctcggcaaggtgaagacccctgtgctgctggtgtcggcggtggacgatcacatcgccctctggcagggcacctggcagggcatgaagctgtttggcggggagcagcgcttcctcctggcggagtccggccacatcgccggcatcatcaacccgccggccgccaacaagtacggcttctggcacaacggggccgaggccgagagcccggagagctggctggcaggggcgacgcaccagggcggctcctggtggcccgagatgatgggctttatccagaaccgtgacgaagggtcagagcccgtccccgcgcgggtcccggaggaagggctggcccccgcccccggccactatgtcaaggtgcggctcaaccccgtgtttgcctgcccaacagaggaggacgccgcatgacctgccggcctggttcaaccagtcggcagccgactagtggatcc

SEQ ID NO: 24 - DNA, 4875 bp, Artificial
  Artificial
tacgctagcgtaccgagctatccatttaaatggagttccagaccctgctcgactttatcgccgaagccgaactggaccgcgtcggctgcttcgcctactcgccggtggagggcgccaccgccaatgacctgccgggcgcgctgcccgacgaggtgcgcgaggaacgccgcgcccgcttcatggaagtggccgaagaggtctcggcgcgccgcctgcagcgcaaggtcggccagaccctgcgcgtgctggtggacgaggtcaaccaggatggcggcatcggccgttcgtccgcggatgcgccggaaatcgacggcctcgtctatatcgcgccgccggaacgccacgcccagcgctatcgcgccggcgagttcgtcgacgtgaagatcaccggcgccgatggccacgacctgtggggcgcggtctgaaacgggttgattaggtaaaagtacgctcgttcgatttcgtccgcgtcccgctatactgtgcggtgcaacataacctcatggagacaaagtccaattggcgcaacgcaattaatgtgagttagctcactcattaggcaccccaggctttacactttatgcttccggctcgtatgttgtgtggaattgtgagcggataacaatttcacacaggaaacaattgcacgtgcagagagacaatcaaatcatgagccaaccatcttatggcccgctgttcgaggccctggcccactacaatgacaagctgctggccatggccaaggcccagacagagcgcaccgcccaggcgctgctgcagaccaatctggacgatctgggccaggtgctggagcagggcagccagcaaccctggcagctgatccaggcccagatgaactggtggcaggatcagctcaagctgatgcagcacaccctgctcaaaagcgcaggccagccgagcgagccggtgatcaccccggagcgcagcgatcgccgcttcaaggccgaggcctggagcgaacaacccatctatgactacctcaagcagtcctacctgctcaccgccaggcacctgctggcctcggtggatgccctggagggcgtcccccagaagagccgggagcggctgcgtttcttcacccgccagtacgtcagcgccatggcccccgccaacttccttgccaccaatcccgaggcgcagcgcctgctgatcgagtcgggcggcgaatcgctgcgtgccggcgtgcgcaacatgatggaagacctgacacgcggcaagatctcgcagaccgacgagagcgcgtttgaggtcggccgcaatgtcgcggtgaccgaaggcgccgtggtcttcgagaacgagtacttccagctgttgcagtacaagccgctgaccgacaaggtgcacgcgcgcccgctgctgatggtgccgccgtgcatcaacaagtactacatcctggacctgcagccggagagctcgctggtgcgccatgtggtggagcagggacatacggtgtttctggtgtcgtggcgcaatccggacgccagcatggccggcagcacctgggacgactacatcgagcacgcggccatccgcgccatcgaagtcgcgcgcgacatcagcggccaggacaagatcaacgtgctcggcttctgcgtgggcggcaccattgtctcgaccgcgctggcggtgctggccgcgcgcggcgagcacccggccgccagcgtcacgctgctgaccacgctgctggactttgccgacacgggcatcctcgacgtctttgtcgacgagggccatgtgcagttgcgcgaggccacgctgggcggcggcgccggcgcgccgtgcgcgctgctgcgcggccttgagctggccaataccttctcgttcttgcgcccgaacgacctggtgtggaactacgtggtcgacaactacctgaagggcaacacgccggtgccgttcgacctgctgttctggaacggcgacgccaccaacctgccggggccgtggtactgctggtacctgcgccacacctacctgcagaacgagctcaaggtaccgggcaagctgaccgtgtgcggcgtgccggtggacctggccagcatcgacgtgccgacctatatctacggctcgcgcgaagaccatatcgtgccgtggaccgcggcctatgcctcgaccgcgctgctggcgaacaagctgcgcttcgtgctgggtgcgtcgggccatatcgccggtgtgatcaacccgccggccaagaacaagcgcagccactggactaacgatgcgctgccggagtcgccgcagcaatggctggccggcgccatcgagcatcacggcagctggtggccggactggaccgcatggctggccgggcaggccggcgcgaaacgcgccgcgcccgccaactatggcaatgcgcgctatcgcgcaatcgaacccgcgcctgggcgatacgtcaaagccaaggcatgacgctttaaagagtgccggcgtgcgtcatgcacggcgccggcaggcctgcaggttccctcccgtttccattgaaaggactacacaatgagccaaccatcttatggcccgctgttcgaggccctggcccactacaatgacaagctgctggccatggccaaggcccagacagagcgcaccgcccaggcgctgctgcagaccaatctggacgatctgggccaggtgctggagcagggcagccagcaaccctggcagctgatccaggcccagatgaactggtggcaggatcagctcaagctgatgcagcacaccctgctcaaaagcgcaggccagccgagcgagccggtgatcaccccggagcgcagcgatcgccgcttcaaggccgaggcctggagcgaacaacccatctatgactacctcaagcagtcctacctgctcaccgccaggcacctgctggcctcggtggatgccctggagggcgtcccccagaagagccgggagcggctgcgtttcttcacccgccagtacgtcagcgccatggcccccagcaacttcctggccaccaaccccgagctgctcaagctgaccctggagtccggcggccagaacctggtgcgcggactggccctcttggccgaggatctggagcgcagcgccgatcagctcaacatccgcctgaccgacgaatccgccttcgagctcgggcgggatctggccctgaccccgggccgggtggtgcagcgcaccgagctctatgagctcattcagtacagcccgactaccgagacggtgggcaagacacctgtgctgatagtgccgcccttcatcaacaagtactacatcatggacatgcggccccagaactccctggtcgcctggctggtcgcccagggccagacggtattcatgatctcctggcgcaacccgggcgtggcccaggcccaaatcgatctcgacgactacgtggtggatggcgtcatcgccgccctggacggcgtggaggcggccaccggcgagcgggaggtgcacggcatcggctactgcatcggcggcaccgccctgtcgctcgccatgggctggctggcggcgcggcgccagaagcagcgggtgcgcaccgccaccctgttcactaccctgctggacttctcccagcccggggagcttggcatcttcatccacgagcccatcatagcggcgctcgaggcgcaaaatgaggccaagggcatcatggacgggcgccagctggcggtctccttcagcctgctgcgggagaacagcctctactggaactactacatcgacagctacctcaagggtcagagcccggtggccttcgatctgctgcactggaacagcgacagcaccaatgtggcgggcaagacccacaacagcctgctgcgccgtctctacctggagaaccagctggtgaagggggagctcaagatccgcaacacccgcatcgatctcggcaaggtgaagacccctgtgctgctggtgtcggcggtggacgatcacatcgccctctggcagggcacctggcagggcatgaagctgtttggcggggagcagcgcttcctcctggcggagtccggccacatcgccggcatcatcaacccgccggccgccaacaagtacggcttctggcacaacggggccgaggccgagagcccggagagctggctggcaggggcgacgcaccagggcggctcctggtggcccgagatgatgggctttatccagaaccgtgacgaagggtcagagcccgtccccgcgcgggtcccggaggaagggctggcccccgcccccggccactatgtcaaggtgcggctcaaccccgtgtttgcctgcccaacagaggaggacgccgcatgacctgccggcctggttcaaccagtcggcagccgactagtggttagccttgcgccttgcttcgctgacgaagaacctctgcgcgctcggcctggccgccgtgctcgcgctggcgggcacggcgcaggcagcgccggcgaccgagctgtcgaccggcccggttaacaccgggccagccggcggcgaaggcctgggcatcaaccaggccattcgcgacggcgaagcccggcgcggcggcacctcgctttccactggcgcgccaaaacccctggcgccgcggccggaatatgcgtcgctgccggtctacgtcggcaaggtcggcgaccagccggtgcggctgcgcctgggccccaagcctgacgagcgcgacagcgtgcgtggcgaatacgccggccgtggcgccggtgtgcgcctgctggcaggcgagtgggaggacggcgccttcctgatggaggagtccgacgacggcacccgcgtatcgggcaactgggaaggcagcatcgacgccagcggcgccgtgcgcggcacctggaccgaatttaaatccgaattcactggccgtcgttttacaacgtcgtgact

SEQ ID NO: 25 - DNA, 4874 bp, Artificial
  Artificial
tacgctagcgtaccgagctatccatttaaatggagttccagaccctgctcgactttatcgccgaagccgaactggaccgcgtcggctgcttcgcctactcgccggtggagggcgccaccgccaatgacctgccgggcgcgctgcccgacgaggtgcgcgaggaacgccgcgcccgcttcatggaagtggccgaagaggtctcggcgcgccgcctgcagcgcaaggtcggccagaccctgcgcgtgctggtggacgaggtcaaccaggatggcggcatcggccgttcgtccgcggatgcgccggaaatcgacggcctcgtctatatcgcgccgccggaacgccacgcccagcgctatcgcgccggcgagttcgtcgacgtgaagatcaccggcgccgatggccacgacctgtggggcgcggtctgaaacgggttgattaggtaaaagtacgctcgttcgatttcgtccgcgtcccgctatactgtgcggtgcaacataacctcatggagacaaagtccaattcgcgcaacgcaattaatgtgagttagctcactcattaggcaccccaggctttacacttatgcttccggctcgtatgttgtgtggaattgtgagcggataacaatttcacacaggaaacaattgcacgtgcagagagacaatcaaatcatgagccaaccatcttatggcccgctgttcgaggccctggcccactacaatgacaagctgctggccatggccaaggcccagacagagcgcaccgcccaggcgctgctgcagaccaatctggacgatctgggccaggtgctggagcagggcagccagcaaccctggcagctgatccaggcccagatgaactggtggcaggatcagctcaagctgatgcagcacaccctgctcaaaagcgcaggccagccgagcgagccggtgatcaccccggagcgcagcgatcgccgcttcaaggccgaggcctggagcgaacaacccatctatgactacctcaagcagtcctacctgctcaccgccaggcacctgctggcctcggtggatgccctggagggcgtcccccagaagagccgggagcggctgcgtttcttcacccgccagtacgtcagcgccatggcccccgccaacttccttgccaccaatcccgaggcgcagcgcctgctgatcgagtcgggcggcgaatcgctgcgtgccggcgtgcgcaacatgatggaagacctgacacgcggcaagatctcgcagaccgacgagagcgcgtttgaggtcggccgcaatgtcgcggtgaccgaaggcgccgtggtcttcgagaacgagtacttccagctgttgcagtacaagccgctgaccgacaaggtgcacgcgcgcccgctgctgatggtgccgccgtgcatcaacaagtactacatcctggacctgcagccggagagctcgctggtgcgccatgtggtggagcagggacatacggtgtttctggtgtcgtggcgcaatccggacgccagcatggccggcagcacctgggacgactacatcgagcacgcggccatccgcgccatcgaagtcgcgcgcgacatcagcggccaggacaagatcaacgtgctcggcttctgcgtgggcggcaccattgtctcgaccgcgctggcggtgctggccgcgcgcggcgagcacccggccgccagcgtcacgctgctgaccacgctgctggactttgccgacacgggcatcctcgacgtctttgtcgacgagggccatgtgcagttgcgcgaggccacgctgggcggcggcgccggcgcgccgtgcgcgctgctgcgcggccttgagctggccaataccttctcgttcttgcgcccgaacgacctggtgtggaactacgtggtcgacaactacctgaagggcaacacgccggtgccgttcgacctgctgttctggaacggcgacgccaccaacctgccggggccgtggtactgctggtacctgcgccacacctacctgcagaacgagctcaaggtaccgggcaagctgaccgtgtgcggcgtgccggtggacctggccagcatcgacgtgccgacctatatctacggctcgcgcgaagaccatatcgtgccgtggaccgcggcctatgcctcgaccgcgctgctggcgaacaagctgcgcttcgtgctgggtgcgtcgggccatatcgccggtgtgatcaacccgccggccaagaacaagcgcagccactggactaacgatgcgctgccggagtcgccgcagcaatggctggccggcgccatcgagcatcacggcagctggtggccggactggaccgcatggctggccgggcaggccggcgcgaaacgcgccgcgcccgccaactatggcaatgcgcgctatcgcgcaatcgaacccgcgcctgggcgatacgtcaaagccaaggcatgacgctttaaagagtgccggcgtgcgtcatgcacggcgccggcaggcctgcaggttccctcccgtttccattgaaaggactacacaatgagccaaccatcttatggcccgctgttcgaggccctggcccactacaatgacaagctgctggccatggccaaggcccagacagagcgcaccgcccaggcgctgctgcagaccaatctggacgatctgggccaggtgctggagcagggcagccagcaaccctggcagctgatccaggcccagatgaactggtggcaggatcagctcaagctgatgcagcacaccctgctcaaaagcgcaggccagccgagcgagccggtgatcaccccggagcgcagcgatcgccgcttcaaggccgaggcctggagcgaacaacccatctatgactacctcaagcagtcctacctgctcaccgccaggcacctgctggcctcggtggatgccctggagggcgtcccccagaagagccgggagcggctgcgtttcttcacccgccagtacgtcagcgccatggcccccagcaacttcctggccaccaaccccgagctgctcaagctgaccctggagtccggcggccagaacctggtgcgcggactggccctcttggccgaggatctggagcgcagcgccgatcagctcaacatccgcctgaccgacgaatccgccttcgagctcgggcgggatctggccctgaccccgggccgggtggtgcagcgcaccgagctctatgagctcattcagtacagcccgactaccgagacggtgggcaagacacctgtgctgatagtgccgcccttcatcaacaagtactacatcatggacatgcggccccagaactccctggtcgcctggctggtcgcccagggccagacggtattcatgatctcctggcgcaacccgggcgtggcccaggcccaaatcgatctcgacgactacgtggtggatggcgtcatcgccgccctggacggcgtggaggcggccaccggcgagcgggaggtgcacggcatcggctactgcatcggcggcaccgccctgtcgctcgccatgggctggctggcggcgcggcgccagaagcagcgggtgcgcaccgccaccctgttcactaccctgctggacttctcccagcccggggagcttggcatcttcatccacgagcccatcatagcggcgctcgaggcgcaaaatgaggccaagggcatcatggacgggcgccagctggcggtctccttcagcctgctgcgggagaacagcctctactggaactactacatcgacagctacctcaagggtcagagcccggtggccttcgatctgctgcactggaacagcgacagcaccaatgtggcgggcaagacccacaacagcctgctgcgccgtctctacctggagaaccagctggtgaagggggagctcaagatccgcaacacccgcatcgatctcggcaaggtgaagacccctgtgctgctggtgtcggcggtggacgatcacatcgccctctggcagggcacctggcagggcatgaagctgtttggcggggagcagcgcttcctcctggcggagtccggccacatcgccggcatcatcaacccgccggccgccaacaagtacggcttctggcacaacggggccgaggccgagagcccggagagctggctggcaggggcgacgcaccagggcggctcctggtggcccgagatgatgggctttatccagaaccgtgacgaagggtcagagcccgtccccgcgcgggtcccggaggaagggctggcccccgcccccggccactatgtcaaggtgcggctcaaccccgtgtttgcctgcccaacagaggaggacgccgcatgacctgccggcctggttcaaccagtcggcagccgactagtggttagccttgcgccttgcttcgctgacgaagaacctctgcgcgctcggcctggccgccgtgctcgcgctggcgggcacggcgcaggcagcgccggcgaccgagctgtcgaccggcccggttaacaccgggccagccggcggcgaaggcctgggcatcaaccaggccattcgcgacggcgaagcccggcgcggcggcacctcgctttccactggcgcgccaaaacccctggcgccgcggccggaatatgcgtcgctgccggtctacgtcggcaaggtcggcgaccagccggtgcggctgcgcctgggccccaagcctgacgagcgcgacagcgtgcgtggcgaatacgccggccgtggcgccggtgtgcgcctgctggcaggcgagtgggaggacggcgccttcctgatggaggagtccgacgacggcacccgcgtatcgggcaactgggaaggcagcatcgacgccagcggcgccgtgcgcggcacctggaccgaatttaaatccgaattcactggccgtcgttttacaacgtcgtgact

SEQ ID NO: 26 - DNA, 3558 bp, Artificial
  Artificial
ggaaacaattgagaaggagatatacatatgattgatcaaaaattcgatccactacaagcatggaaaaatgcttatgaacaaaccgaaacattttggggaaaagcgctcaatgaaacaattaaaacagaagaatattctgcttggatgggcagcgttctagatttgaatttgttttatcaaaaagcattaaatgatacgacaaaaaattatttagagcaggtgaatgtgcctacgaaagaggatatcgctagagtggctacgcttgttattaacttagaaaataaagtggataacattgaggagtttctagaagagaaggtagagtcagtaggacaagctcctacattaaagcgcgatgttacgaaagtaaaacaagatattcgcacattagaaacgaaagttgatcaaattttagaattgctagaaaagcaaaatgcagtactagcaaaactacaagaacctgtaaaagaagaagtaaaacctacgaataagccagaaaataaaaagtgataatagcgcttgtttataacttatgaaagacctgcaggagaaggagatatacatatgactacattcgcaacagaatgggaaaagcaattagagctatacccagaagagtaccgaaaagcatatcgccgagtgaaaagggcgagtgaaattttattacgtgaaccagagccacaagtaggattaacgccgaaagaggttatttggacgaagaataagacgaagctttatcgctacattccaaaacaagaaaaaacacaaagagttccaattctattaatatatgctcttattaataaaccatatattatggatttaactcctggaaatagtttagtggaatatctagtggaccgtggttttgatgtgtatatgcttgattggggcacatttggtttagaagatagtcatttgaaatttgatgattttgtgtttgattatattgcaaaagcagtgaaaaaagtaatgcgaactgcaaaatcggacgagatttctttacttggttattgcatggggggaacgctaacttctatttatgcggcacttcatccacacatgccaattcgtaacctaatctttatgacaagtccttttgatttctctgaaacaggattatatggtcctttattagacgagaaatacttcaatctagataaagcggttgatacatttggaaacattccgccagaaatgattgatttcggaaacaaaatgttaaaaccaattacaaactttgttggtccatatgttgctttagtagatcgttcagagaatgagcgcttcgtcgaaagctggagattggttcaaaagtgggttggtgatggtattccgttcccaggtgaatcatacagacagtggattcgtgatttttatcaaaataataaattggttaagggtgaacttgtgattcgcggacaaaaagtagaccttgcaaatattaaggcgaatgtcttaaatatttccgggaaacgtgatcatatcgctttgccatgtcaagtagaagcattactagaccatatttctagcacagataaacaatatgtatgtttaccgacagggcatatgtctatcgtttacggtggaacagctgtaaaacaaacatatccgacgattggaaattggcttgaagagcgttctaattaatttaaagagtgccggcgtgcgtcatgcacggcgccggcaggcctgcaggttccctcccgtttccattgaaaggactacacaatgagccaaccatcttatggcccgctgttcgaggccctggcccactacaatgacaagctgctggccatggccaaggcccagacagagcgcaccgcccaggcgctgctgcagaccaatctggacgatctgggccaggtgctggagcagggcagccagcaaccctggcagctgatccaggcccagatgaactggtggcaggatcagctcaagctgatgcagcacaccctgctcaaaagcgcaggccagccgagcgagccggtgatcaccccggagcgcagcgatcgccgcttcaaggccgaggcctggagcgaacaacccatctatgactacctcaagcagtcctacctgctcaccgccaggcacctgctggcctcggtggatgccctggagggcgtcccccagaagagccgggagcggctgcgtttcttcacccgccagtacgtcagcgccatggcccccagcaacttcctggccaccaaccccgagctgctcaagctgaccctggagtccggcggccagaacctggtgcgcggactggccctcttggccgaggatctggagcgcagcgccgatcagctcaacatccgcctgaccgacgaatccgccttcgagctcgggcgggatctggccctgaccccgggccgggtggtgcagcgcaccgagctctatgagctcattcagtacagcccgactaccgagacggtgggcaagacacctgtgctgatagtgccgcccttcatcaacaagtactacatcatggacatgcggccccagaactccctggtcgcctggctggtcgcccagggccagacggtattcatgatctcctggcgcaacccgggcgtggcccaggcccaaatcgatctcgacgactacgtggtggatggcgtcatcgccgccctggacggcgtggaggcggccaccggcgagcgggaggtgcacggcatcggctactgcatcggcggcaccgccctgtcgctcgccatgggctggctggcggcgcggcgccagaagcagcgggtgcgcaccgccaccctgttcactaccctgctggacttctcccagcccggggagcttggcatcttcatccacgagcccatcatagcggcgctcgaggcgcaaaatgaggccaagggcatcatggacgggcgccagctggcggtcaccttcagcctgctgcgggagaacagcctctactggaactactacatcgacagctacctcaagggtcagagcccggtggccttcgatctgctgcactggaacagcgacagcaccaatgtggcgggcaagacccacaacagcctgctgcgccgtctctacctggagaaccagctggtgaagggggagctcaagatccgcaacacccgcatcgatctcggcaaggtgaagacccctgtgctgctggtgtcggcggtggacgatcacatcgccctctggcagggcacctggcagggcatgaagctgtttggcggggagcagcgcttcctcctggcggagtccggccacatcgccggcatcatcaacccgccggccgccaacaagtacggcttctggcacaacggggccgaggccgagagcccggagagctggctggcaggggcgacgcaccagggcggctcctggtggcccgagatgatgggctttatccagaaccgtgacgaagggtcagagcccgtccccgcgcgggtcccggaggaagggctggcccccgcccccggccactatgtcaaggtgcggctcaaccccgtgtttgcctgcccaacagaggaggacgccgcatgacctgccggcctggttcaaccagtcggcagccgactagtggat

SEQ ID NO: 27 - DNA, 2771 bp, Artificial
  Artificial
tacgctagcgtaccgagctatccatttaaattgcatgcgggcttgcacgtgccgcatgcgcggctggtgatccgcaagggccaccatgccgacgtggacagctactccgccttcctggaggcggaccgcaccacgcgcaccgggctggccggctacctgcgcgagcatggcgtcaggcgcgtgttctgcgcgggtctggcgacggactactgcgtggcctggagcgcgctcgatgcacgcgccgcgggcttcgcggccgcggtgatcgaggatgcctgccgcgccatcgacctggaagggtcgctggccaaagcatggcaggacctcggcgccgccggcgttgcgcgcgtcacgtccgctgaactgctcaagggccagggctgaaccgaaccaccgaactgaacgacacaagagaatccgaggagcaagaccaattcgcgcaacgcaattaatgtgagttagctcactcattaggcaccccaggctttacacttatgcttccggctcgtatgttgtgtggaattgtgagcggataacaatttcacacaggaaacaattccacgtgcagagagacaatcaaatcatgcagcagtttgtcaattccctgtcgctcggccaggaccagtccgatgccccccatccgctgaccggcgcctggtcgcagctgatgagccagaccaatcagctcttgcagctgcaatccagcctctaccaacagcaattgggcttgtggacgcaattcctcggccaaaccgccggcaacgacgcttccgcgccgtcggccaagccgagcgaccgccgcttcgcctcgccggagtgggatgagcatccgttctacagcttcctcaagcagagctatctgcaaacctccaagtggatgatggagctggtggacaagacccagatcgacgaaagcgctaaggacaagctgtccttcgccactcgccagtacctggatgccatggcgcccagcaacttcatgctgaccaaccccgacgtggtcaaacgcgccatcgaaacccagggcgaaagcctggtggaaggcatgaagaacatgatggaggacatccagaagggccatatctcgatgtccgacgagagcaagttccaaatcggcaaaaacctggtggtgacgccgggcgaggtggtgttccgcaatgaactgatcgagctgatccagtacacgccgaccaccgaaaaagtccacgaaaagcccttgctgtttgtcccgccgtgcatcaacaagtactacctgatggatctgcagccggacaactccatggtgcgccacttcgtcggccagggttaccgcgttttcctggtcagctggcgttccgccgtgcccgagatgaagaacttcacttgggagacctacatcgagaaaggcgtgttcgccgcggccgaagcggttcagaagatcaccaagcagccgaccatgaacgcgctgggcttctgcgtgggcggcgtgatcctcactaccgcgctgtgcgtggcccaggccaagggtctgaaatacttcgactccgccaccttcatgacgtcgctgatcgaccacgccgaaccgggcgagatctccttcttcatcgacgaggcgctggtagccagccgcgaagccaaaatggcggccggcggcatcatcagcggcaaggaaatcggacgcactttcgccagcctgcgcgccaacgacctggtgtggaactacgtcgtcaacaactacctgctgggcaagaccccggcgccgttcgacctgctgtactggaacaacgacgcggtggacctgccgctgccgatgcacaccttcatgctgcggcagttctacatcaacaacgcgctgatcaccccgggcgccattacgctgtgcggcgtcccgatcgacatctccaagatcgacatcccggtgtatatgttcgccgcgcgcgaagaccacatcgtgctgtggagttccgcctactccggcctgaaatatctgagcggcacgccaagccgccgctttgtcctgggcgcatccggccacatcggcggctcgatcaaccccgtcaccaaggataagcgcaactactggaccaacgagcagctgccggtgaatccggaagaatggctggagggcgcgcaaagccatccaggcagctggtggaaggactgggacgcctggctggccccgcaatccggaaaacaggttccggcgcccaagatgctgggcagcaaggagttccccccgctgcagcctgcgccgggcagctatgtgctcgccaaggcgatgcctcccgtcgccgccgccttgaactgacctgccggcctggttcaaccagtcggcagccgactagtatgtcggctgcgggcaccgcgcgggccacgcccgccgacatgctcgcctggggccgggaggtgctggccagccagcccttctcggtcctggtcggcaccgaactggcggcgttgtcgccgggcaaggctgagttgcgcctgccgatccgtcaggacctgcggcagcagcacggcttcctgcacggcggcgtggtcagctacctggccgacaatgcgctgacctacgcgggcggcgcggccatggcggtgccggtcgtgacatccgagtacaagatcaactacgtgcgcccggcgatcggcgagctgctggtcgcccgcgccgaatgcgtcagcgccggccgccagcaggcggtggtgcgctgcgacgtgtacgtcgtcagggatggcgaggagaggctctgatttaaatccgaattcactggccgtcgttttacaacgtcgtgact

SEQ ID NO: 28 - DNA, 3034 bp, Artificial
  Artificial
gcgcatttaaatccggaccttcgtgcggctcaagccccagcacgtcgccgggcagcgaaaaacccgttacctgccgccagcccagcggcgattcatagacctgcttggcgctgccatggcgcagcgggtagaccgtcagcgcagggcggccctggcgaaacacatgctcgccggtgcgcacctctaccagctccggctgcagcgccatcggcgcgtgcggcaggggggcttgtggcccggcattgtggcaaacgtggcgaaagaggcagagcaggcaggctggggcgccgctgtccggcatggtgtcattgtcctccggtgacgatggccaagtataaaacgccggcaacgcaagccatctcgctgcgatctgcattctttcgtatggctggtttaaaaatttcgcattacgggggcgaggctcgttgcgtttgtgccataagcgcgggagcacgccggcgggcgtaatgcggattgtgatatgctgcaacgcaacaataaaggcataggaggagatcgcgtcacacgatcaggagtcctccaattggcgcaacgcaattaatgtgagttagctcactcattaggcaccccaggctttacacttatgcttccggctcgtatgttgtgtggaattgtgagcggataacaatttcacacaggaaacaattgcacgtgcagagagacaatcaaatcatgagccaaccatcttatggcccgctgttcgaggccctggcccactacaatgacaagctgctggccatggccaaggcccagacagagcgcaccgcccaggcgctgctgcagaccaatctggacgatctgggccaggtgctggagcagggcagccagcaaccctggcagctgatccaggcccagatgaactggtggcaggatcagctcaagctgatgcagcacaccctgctcaaaagcgcaggccagccgagcgagccggtgatcaccccggagcgcagcgatcgccgcttcaaggccgaggcctggagcgaacaacccatctatgactacctcaagcagtcctacctgctcaccgccaggcacctgctggcctcggtggatgccctggagggcgtcccccagaagagccgggagcggctgcgtttcttcacccgccagtacgtcagcgccatggcccccagcaacttcctggccaccaaccccgagctgctcaagctgaccctggagtccggcggccagaacctggtgcgcggactggccctcttggccgaggatctggagcgcagcgccgatcagctcaacatccgcctgaccgacgaatccgccttcgagctcgggcgggatctggccctgaccccgggccgggtggtgcagcgcaccgagctctatgagctcattcagtacagcccgactaccgagacggtgggcaagacacctgtgctgatagtgccgcccttcatcaacaagtactacatcatggacatgcggccccagaactccctggtcgcctggctggtcgcccagggccagacggtattcatgatctcctggcgcaacccgggcgtggcccaggcccaaatcgatctcgacgactacgtggtggatggcgtcatcgccgccctggacggcgtggaggcggccaccggcgagcgggaggtgcacggcatcggctactgcatcggcggcaccgccctgtcgctcgccatgggctggctggcggcgcggcgccagaagcagcgggtgcgcaccgccaccctgttcactaccctgctggacttctcccagcccggggagcttggcatcttcatccacgagcccatcatagcggcgctcgaggcgcaaaatgaggccaagggcatcatggacgggcgccagctggcggtctccttcagcctgctgcgggagaacagcctctactggaactactacatcgacagctacctcaagggtcagagcccggtggccttcgatctgctgcactggaacagcgacagcaccaatgtggcgggcaagacccacaacagcctgctgcgccgtctctacctggagaaccagctggtgaagggggagctcaagatccgcaacacccgcatcgatctcggcaaggtgaagacccctgtgctgctggtgtcggcggtggacgatcacatcgccctctggcagggcacctggcagggcatgaagctgtttggcggggagcagcgcttcctcctggcggagtccggccacatcgccggcatcatcaacccgccggccgccaacaagtacggcttctggcacaacggggccgaggccgagagcccggagagctggctggcaggggcgacgcaccagggcggctcctggtggcccgagatgatgggctttatccagaaccgtgacgaagggtcagagcccgtccccgcgcgggtcccggaggaagggctggcccccgcccccggccactatgtcaaggtgcggctcaaccccgtgtttgcctgcccaacagaggaggacgccgcatgagcctgacctgccggcctggttcaaccagtcggcagccgactagtagtcgggcagcaccaatgcgcatcaagcgcgcacaagtaaagggagggcgcctgccctccctttttccttgcagcagccgcgtcagccgcgcgagcggtccttgacgaacagcgcagtcaccatgcccagcacgcacagcgcgaccacatagtgggccggtgccagcggatcctgcttcagcatcagcgtgacgaccatcggcgtcagcccgccgaagatcgcatacgacacgttgtacgagaatgacaggcccgagaagcgcacctgcgccgggaacgcattgaccagcacgaacggcaccgcgccgatggtgccgaccaggaagccggtcagcgcatagagcggcagcagcaggtcggggcgggtgaagatcgtcgtgtagaacatataggcgcagatggccagcagcaggccgccgacgaacagcgtgcggcgcgcaccgatgcggtcggctaatgcgccggagacgacacagccgatcgtcaggcacagcgtggcgatttaaatgcgc

SEQ ID NO: 29 - DNA, 2841 bp, Artificial
  Artificial
gcgcgcatttaaatctgccaccacgttgtgctcggtgatcgccatcatcagcgccacgtagagccagccaatggccacgatgtacatcaaaaattcatccttctcgcctatgctctggggcctcggcagatgcgagcgctgcataccgtccggtaggtcgggaagcgtgcagtgccgaggcggattcccgcattgacagcgcgtgcgttgcaaggcaacaatggactcaaatgtctcggaatcgctgacgattcccaggtttctccggcaagcatagcgcatggcgtctccatgcgagaatgtcgcgcttgccggataaaaggggagccgctatcggaatggacgcaagccacggccgcagcaggtgcggtcgagggcttccagccagttccagggcagatgtgccggcagaccctcccgctttgggggaggcgcaagccgggtccattcggatagcatctccccatgcaaagtgccggccagggcaatgcccggagccggttcgaatagtgacggcagagagacaatcaaatcatgagccaaccatcttatggcccgctgttcgaggccctggcccactacaatgacaagctgctggccatggccaaggcccagacagagcgcaccgcccaggcgctgctgcagaccaatctggacgatctgggccaggtgctggagcagggcagccagcaaccctggcagctgatccaggcccagatgaactggtggcaggatcagctcaagctgatgcagcacaccctgctcaaaagcgcaggccagccgagcgagccggtgatcaccccggagcgcagcgatcgccgcttcaaggccgaggcctggagcgaacaacccatctatgactacctcaagcagtcctacctgctcaccgccaggcacctgctggcctcggtggatgccctggagggcgtcccccagaagagccgggagcggctgcgtttcttcacccgccagtacgtcagcgccatggcccccagcaacttcctggccaccaaccccgagctgctcaagctgaccctggagtccggcggccagaacctggtgcgcggactggccctcttggccgaggatctggagcgcagcgccgatcagctcaacatccgcctgaccgacgaatccgccttcgagctcgggcgggatctggccctgaccccgggccgggtggtgcagcgcaccgagctctatgagctcattcagtacagcccgactaccgagacggtgggcaagacacctgtgctgatagtgccgcccttcatcaacaagtactacatcatggacatgcggccccagaactccctggtcgcctggctggtcgcccagggccagacggtattcatgatctcctggcgcaacccgggcgtggcccaggcccaaatcgatctcgacgactacgtggtggatggcgtcatcgccgccctggacggcgtggaggcggccaccggcgagcgggaggtgcacggcatcggctactgcatcggcggcaccgccctgtcgctcgccatgggctggctggcggcgcggcgccagaagcagcgggtgcgcaccgccaccctgttcactaccctgctggacttctcccagcccggggagcttggcatcttcatccacgagcccatcatagcggcgctcgaggcgcaaaatgaggccaagggcatcatggacgggcgccagctggcggtcaccttcagcctgctgcgggagaacagcctctactggaactactacatcgacagctacctcaagggtcagagcccggtggccttcgatctgctgcactggaacagcgacagcaccaatgtggcgggcaagacccacaacagcctgctgcgccgtctctacctggagaaccagctggtgaagggggagctcaagatccgcaacacccgcatcgatctcggcaaggtgaagacccctgtgctgctggtgtcggcggtggacgatcacatcgccctctggcagggcacctggcagggcatgaagctgtttggcggggagcagcgcttcctcctggcggagtccggccacatcgccggcatcatcaacccgccggccgccaacaagtacggcttctggcacaacggggccgaggccgagagcccggagagctggctggcaggggcgacgcaccagggcggctcctggtggcccgagatgatgggctttatccagaaccgtgacgaagggtcagagcccgtccccgcgcgggtcccggaggaagggctggcccccgcccccggccactatgtcaaggtgcggctcaaccccgtgtttgcctgcccaacagaggaggacgccgcatgacgcttgcatgagtgccggcgtgcgtcatgcacagcgccggcaggcctgcaggttccctcccgtttccattgaaaggactacacaatgactgacgttgtcatcgtatccgccgcccgcaccgcggtcggcaagtttggcggctcgctggccaagatcccggcaccggaactgggtgccgtggtcatcaaggccgcgctggagcgcgccggcgtcaagccggagcaggtgagcgaagtcatcatgggccaggtgctgaccgccggttcgggccagaaccccgcacgccaggccgcgatcaaggccggcctgccggcgatggtgccggccatgaccatcaacaaggtgtgcggctcgggcctgaaggccgtgatgctggccgccaacgcgatcatggcgggcgacgccgagatcgtggtggccggcggccaggaaaacatgagcgccgccccgcacgtgctgccgggctcgcgcgatggtttccgcatgggcgatgccaagctggtcgacaatttaaatgcgcgc

SEQ ID NO: 30 - DNA, 1864 bp, Artificial
  Artificial
ggaaacaattgcacgtgcagagagacaatcaaatcatgagccaaccatcttatggcccgctgttcgaggccctggcccactacaatgacaagctgctggccatggccaaggcccagacagagcgcaccgcccaggcgctgctgcagaccaatctggacgatctgggccaggtgctggagcagggcagccagcaaccctggcagctgatccaggcccagatgaactggtggcaggatcagctcaagctgatgcagcacaccctgctcaaaagcgcaggccagccgagcgagccggtgatcaccccggagcgcagcgatcgccgcttcaaggccgaggcctggagcgaacaacccatctatgactacctcaagcagtcctacctgctcaccgccaggcacctgctggcctcggtggatgccctggagggcgtcccccagaagagccgggagcggctgcgtttcttcacccgccagtacgtcagcgccatggcccccagcaacttcctggccaccaaccccgagctgctcaagctgaccctggagtccggcggccagaacctggtgcgcggactggccctcttggccgaggatctggagcgcagcgccgatcagctcaacatccgcctgaccgacgaatccgccttcgagctcgggcgggatctggccctgaccccgggccgggtggtgcagcgcaccgagctctatgagctcattcagtacagcccgactaccgagacggtgggcaagacacctgtgctgatagtgccgcccttcatcaacaagtactacatcatggacatgcggccccagaactccctggtcgcctggctggtcgcccagggccagacggtattcatgatctcctggcgcaacccgggcgtggcccaggcccaaatcgatctcgacgactacgtggtggatggcgtcatcgccgccctggacggcgtggaggcggccaccggcgagcgggaggtgcacggcatcggctactgcatcggcggcaccgccctgtcgctcgccatgggctggctggcggcgcggcgccagaagcagcgggtgcgcaccgccaccctgttcactaccctgctggacttctcccagcccggggagcttggcatcttcatccacgagcccatcatagcggcgctcgaggcgcaaaatgaggccaagggcatcatggacgggcgccagctggcggtcaccttcagcctgctgcgggagaacagcctctactggaactactacatcgacagctacctcaagggtcagagcccggtggccttcgatctgctgcactggaacagcgacagcaccaatgtggcgggcaagacccacaacagcctgctgcgccgtctctacctggagaaccagctggtgaagggggagctcaagatccgcaacacccgcatcgatctcggcaaggtgaagacccctgtgctgctggtgtcggcggtggacgatcacatcgccctctggcagggcacctggcagggcatgaagctgtttggcggggagcagcgcttcctcctggcggagtccggccacatcgccggcatcatcaacccgccggccgccaacaagtacggcttctggcacaacggggccgaggccgagagcccggagagctggctggcaggggcgacgcaccagggcggctcctggtggcccgagatgatgggctttatccagaaccgtgacgaagggtcagagcccgtccccgcgcgggtcccggaggaagggctggcccccgcccccggccactatgtcaaggtgcggctcaaccccgtgtttgcctgcccaacagaggaggacgccgcatgacctgccggcctggttcaaccagtcggcagccgactagtgcgcgc

SEQ ID NO: 31 - DNA, 246 bp, Artificial
  Artificial
gcgccaattgtgcttctggcgtcaggcagccatcggaagctgtggtatggctgtgcaggtcgtaaatcactgcataattcgtgtcgctcaaggcgcactcccgttctggataatgttttttgcgccgacatcataacggttctggcaaatattctgaaatgagctgttgacaattaatcatcgaactagttaactagtacgcaagttcacagcggataacaatttcacacaggaaacaattggcgc